European Patent Application EP 4 293 036 A2, published December 20, 2023. Title: STRUCTURE OF GII.4 NOROVIRUS PROTEASE - DESIGN OF BROAD-SPECTRUM PROTEASE INHIBITORS. Applicant: BAYLOR COLLEGE OF MEDICINE. Application EP 23190471.5, filed October 5, 2017. The sequence listing filed with the application follows.

SEQUENCE LISTING (2 sequences)

SEQ ID NO: 1 - protein, 180 aa, Houston virus
APPSIWSRIVNFGSGWGFWVSPSLFITSTHVIPQGAKEFFGVPIKQIQVHKSGEFCRLRFPKPIRTDVTGMILEEGAPEGTVVTLLIKRSTGELMPLAARMGTHATMKIQGRTVGGQMGMLLTGSNAKSMDLGTTPGDCGCPYIYKRGNDYVVIGVHTAAARGGNTVICATQGSEGEATL

SEQ ID NO: 2 - protein, 180 aa, Norwalk virus
APPTLWSRVTKFGSGWGFWVSPTVFITTTHVVPTGVKEFFGEPLSSIAIHQAGEFTQFRFSKKMRPDLTGMVLEEGCPEGTVCSVLIKRDSGELLPLAVRMGAIASMRIQGRLVHGQSGMLLTGANAKGMDLGTIPGDCGAPYVHKRGNDWVVCGVHAAATKSGNTVVCAVQAGEGETAL